European Patent Application EP 4 116 330 A1, published January 11, 2023. Title: Multispecific antibodies with monovalent binding to tumor-associated antigens causing no or reduced nerve pain in the treatment of cancer. Applicant: Trion Research GmbH. The sequence listing filed with the application follows.

SEQUENCE LISTING (4 sequences)

SEQ ID NO: 1 - protein, 6 aa, artificial
  complement binding motif of Fc-portion
EELGGP

SEQ ID NO: 2 - protein, 6 aa, artificial
  complement binding motif of Fc-portion
EFLGGP

SEQ ID NO: 3 - protein, 6 aa, artificial
  complement binding motif of Fc-portion
PVAGGP

SEQ ID NO: 4 - protein, 3 aa, artificial
  substituted complement binding motif of Fc-portion
PVA